European Patent Application EP 4 596 689 A1, published August 6, 2025. Title: Enzyme agents and their application. Applicant: AMANO ENZYME INC. The sequence listing filed with the application follows.

SEQUENCE LISTING (14 sequences)

SEQ ID NO: 1 - protein, 431 aa, Aspergillus nidulans
AETMEYLMSLKQQSRERARSQGLFDINRYPDEGAKKCKNGKAGEYSCENVDLLSFLSHQALGSVTREGNDVWGWTSAEGREFGIVGQTDGVAFVEILEDGSLEYVGRLGSQTEPSTWRDIKVIGDHAYIGSEAAGHGLQIFDLNKLTTASSSKPTVFSTKKDLTAWYRGFGSSHNIVAHEETNMIYAVGTARNLSCAGGLWMVDVSDPANPTSPGCVNEDGYVHDAQCVIYKGPDEKYIGQEICFNFNEDTLTIADVTDKKNPIQISKTPYVGASYTHQGWLVDENDHSYLLLDDELDEMDGTGSAANGHTTTYIFDIKDLSAPKHTGTYQSPVRSIDHNQYVVAGLSYQSNYGSGLRVVDVSSVFEDPTASSFKEVGSFDVHPEDDAVGGEVEFVGSWSVYPFFASGHILLNSIERGIYSLKYTGPAAEN

SEQ ID NO: 2 - protein, 452 aa, Aspergillus nidulans
MKLSALSLLTVACVATASSHGAETMEYLMSLKQQSRERARSQGLFDINRYPDEGAKKCKNGKAGEYSCENVDLLSFLSHQALGSVTREGNDVWGWTSAEGREFGIVGQTDGVAFVEILEDGSLEYVGRLGSQTEPSTWRDIKVIGDHAYIGSEAAGHGLQIFDLNKLTTASSSKPTVFSTKKDLTAWYRGFGSSHNIVAHEETNMIYAVGTARNLSCAGGLWMVDVSDPANPTSPGCVNEDGYVHDAQCVIYKGPDEKYIGQEICFNFNEDTLTIADVTDKKNPIQISKTPYVGASYTHQGWLVDENDHSYLLLDDELDEMDGTGSAANGHTTTYIFDIKDLSAPKHTGTYQSPVRSIDHNQYVVAGLSYQSNYGSGLRVVDVSSVFEDPTASSFKEVGSFDVHPEDDAVGGEVEFVGSWSVYPFFASGHILLNSIERGIYSLKYTGPAAEN

SEQ ID NO: 3 - DNA, 1296 bp, synthetic construct
  source 1..1296: mol_type = other DNA
gccgagacaatggagtatctcatgtccctgaagcagcaatctcgagaacgtgcccgttcacagggtctgtttgatatcaaccgctaccccgacgagggagccaagaagtgcaagaacggcaaggcaggagagtactcctgcgagaacgtcgacctcttgtccttcctcagtcaccaggctttgggtagtgtcacccgtgagggtaacgacgtctggggctggacttctgctgaaggtcgcgagtttggcattgtcggccagactgacggcgtggcctttgttgagattctggaggacggtagcctcgaatatgttggccgcctgggttctcaaacggaaccatccacgtggcgcgatatcaaggttatcggtgaccatgcctacattggctccgaggctgcagggcatgggctgcagattttcgacctcaacaagttgacaactgcgtctagctcaaagccgaccgttttctccacaaagaaggacttgaccgcgtggtataggggcttcggaagctctcataatatcgttgcgcacgaggagaccaatatgatctatgctgttggaacagcccgcaacctcagctgcgccggaggcctgtggatggtcgatgtgtctgacccagccaaccctacctcgccgggttgtgtcaacgaagatggttatgtgcatgatgcccaatgcgtcatttacaagggccccgatgagaaatatatcggtcaggagatctgcttcaactttaacgaggacacactcaccattgccgacgtaaccgacaagaagaacccaattcagatctcgaagaccccctacgtcggcgccagctacactcaccagggctggctcgttgacgaaaacgaccattcctacctcctcctcgacgacgagctcgacgaaatggacggaacgggctccgccgctaacggccacaccaccacctacatcttcgacatcaaggatctctctgcacccaagcacactggtacctaccagtcccccgtccgctcaatcgaccacaaccagtatgttgtcgcgggtctctcttaccagtccaactacggcagcggtctgcgtgtcgtcgatgtcagctctgtctttgaggaccccacggcatctagcttcaaggaagtcggctctttcgacgtccaccccgaggatgatgcggttggcggtgaggtggagtttgtcggaagctggagtgtttacccgttctttgcgagcgggcatatcttgctcaacagtattgagcgcggcatttactctctcaagtataccggcccagccgcggagaactag

SEQ ID NO: 4 - DNA, 1359 bp, synthetic construct
  source 1..1359: mol_type = other DNA
atgaagctctcggccctatctctgctcaccgtggcctgtgtggcaacagcgtcaagtcatggcgccgagacaatggagtatctcatgtccctgaagcagcaatctcgagaacgtgcccgttcacagggtctgtttgatatcaaccgctaccccgacgagggagccaagaagtgcaagaacggcaaggcaggagagtactcctgcgagaacgtcgacctcttgtccttcctcagtcaccaggctttgggtagtgtcacccgtgagggtaacgacgtctggggctggacttctgctgaaggtcgcgagtttggcattgtcggccagactgacggcgtggcctttgttgagattctggaggacggtagcctcgaatatgttggccgcctgggttctcaaacggaaccatccacgtggcgcgatatcaaggttatcggtgaccatgcctacattggctccgaggctgcagggcatgggctgcagattttcgacctcaacaagttgacaactgcgtctagctcaaagccgaccgttttctccacaaagaaggacttgaccgcgtggtataggggcttcggaagctctcataatatcgttgcgcacgaggagaccaatatgatctatgctgttggaacagcccgcaacctcagctgcgccggaggcctgtggatggtcgatgtgtctgacccagccaaccctacctcgccgggttgtgtcaacgaagatggttatgtgcatgatgcccaatgcgtcatttacaagggccccgatgagaaatatatcggtcaggagatctgcttcaactttaacgaggacacactcaccattgccgacgtaaccgacaagaagaacccaattcagatctcgaagaccccctacgtcggcgccagctacactcaccagggctggctcgttgacgaaaacgaccattcctacctcctcctcgacgacgagctcgacgaaatggacggaacgggctccgccgctaacggccacaccaccacctacatcttcgacatcaaggatctctctgcacccaagcacactggtacctaccagtcccccgtccgctcaatcgaccacaaccagtatgttgtcgcgggtctctcttaccagtccaactacggcagcggtctgcgtgtcgtcgatgtcagctctgtctttgaggaccccacggcatctagcttcaaggaagtcggctctttcgacgtccaccccgaggatgatgcggttggcggtgaggtggagtttgtcggaagctggagtgtttacccgttctttgcgagcgggcatatcttgctcaacagtattgagcgcggcatttactctctcaagtataccggcccagccgcggagaactag

SEQ ID NO: 5 - DNA, 1500 bp, Aspergillus nidulans
  source 1..1500: mol_type = genomic DNA
atgaagctctcggccctatctctgctcaccgtggcctgtgtggcaacagcgtcaagtcatggcgccgagacaatggagtatctcatgtccctgaagcagcaatctcgagaacgtgcccgttcacagggtctgtttgatatcaaccgctaccccgacgagggagccaagaagtgcaagaacggcaaggcaggagagtactcctgcgagaacgtcgacctcttgtccttcctcagtcaccaggctttgggtagtgtcacccgtgagggtaacgacgtctggggtgagcactcaacgtccctcaccaagggctgagctaaccgacgtaggctggacttctgctgaaggtcgcgagtttggcattgtcggccagactgacggcgtggcctttgttgagattctggaggacggtagcctcgaatatgttggccgcctgggttctcaaacggaaccatccacgtggcgcgatatcaaggttatcggtgaccatgcctacattggctccgaggctgcagggcatgggctgcagattttcgacctcaacaaggtatggtagcttcccaatttataacgagcgtctgctgacagccatagttgacaactgcgtctagctcaaagccgaccgttttctccacaaagaaggacttgaccgcgtggtataggggcttcggaagctctcataatatcgttgcgcacgaggagaccaatatgatctatgctgttggaacagcccgcaacctcagctgcgccggaggcctgtggatggtcgatgtgtctgacccagccaaccctacctcgccgggttgtgtcaacgaagatggttatgtgcatgatggtaggttgagggatctccgcagttgagaacacgagctgacctactcagcccaatgcgtcatttacaagggccccgatgagaaatatatcggtcaggagatctgcttcaactttaacgaggacacactcaccattgccgacgtaaccgacaagaagaacccaattcagatctcgaagaccccctacgtcggcgccagctacactcaccagggctggctcgttgacgaaaacgaccattcctacctcctcctcgacgacgagctcgacgaaatggacggaacgggctccgccgctaacggccacaccaccacctacatcttcgacatcaaggatctctctgcacccaagcacactggtacctaccagtcccccgtccgctcaatcgaccacaaccagtatgttgtcgcgggtctctcttaccagtccaactacggcagcggtctgcgtgtcgtcgatgtcagctctgtctttgaggaccccacggcatctagcttcaaggaagtcggctctttcgacgtccaccccgaggatgatgcggttggcggtgaggtggagtttgtcggaagctggagtgtttacccgttctttgcgagcgggcatatcttgctcaacagtattgagcgcggcatttactctctcaagtataccggcccagccgcggagaactag

SEQ ID NO: 6 - protein, 5 aa, synthetic construct
AAAAA

SEQ ID NO: 7 - protein, 10 aa, synthetic construct
KRPPGFSPFR

SEQ ID NO: 8 - protein, 427 aa, Aspergillus oryzae
APIMSHLMSIKTEHRERARAQGLFKPNSYIDLAKTPCVDGKAGEYSCENVDLLGFLSHQAMGSTTREGNDIWGWTSADGREFGIVGQTDGTAFVEVLDDGSLQYVGRLPTQTTATIWRDMKVIGDHAYIGSESPGHGLQIFDLKKLLETDSNNPTNFSTTEDLTAWYSGFGSSHNIVAHEETNMIFAVGTARNLSCAGGLWMIDVSDPANPTSPGCVSEDGYVHDAQCVIYTGPDKEYTNREICFNYNEDTLTIVDITDRASPIQISKTPYVGASYTHQGWIAVSDMSYLLLDDELDEQDGTGEAANGHTTTYIFDIKDLANPKHTGTYQSPVRSIDHNQYVIDGLTYQANYGSGLRIVDVSSVKDDPTGKGFKQVGFFDCHPEDDAQGGEVEFVGAWSVYPYFRSGNILLNSIERGVYSLKYTGKA

SEQ ID NO: 9 - protein, 448 aa, Aspergillus oryzae
MKPSFVSLLSLACLGAASREGAPIMSHLMSIKTEHRERARAQGLFKPNSYIDLAKTPCVDGKAGEYSCENVDLLGFLSHQAMGSTTREGNDIWGWTSADGREFGIVGQTDGTAFVEVLDDGSLQYVGRLPTQTTATIWRDMKVIGDHAYIGSESPGHGLQIFDLKKLLETDSNNPTNFSTTEDLTAWYSGFGSSHNIVAHEETNMIFAVGTARNLSCAGGLWMIDVSDPANPTSPGCVSEDGYVHDAQCVIYTGPDKEYTNREICFNYNEDTLTIVDITDRASPIQISKTPYVGASYTHQGWIAVSDMSYLLLDDELDEQDGTGEAANGHTTTYIFDIKDLANPKHTGTYQSPVRSIDHNQYVIDGLTYQANYGSGLRIVDVSSVKDDPTGKGFKQVGFFDCHPEDDAQGGEVEFVGAWSVYPYFRSGNILLNSIERGVYSLKYTGKA

SEQ ID NO: 10 - DNA, 1284 bp, synthetic construct
  source 1..1284: mol_type = other DNA
gctccgattatgagccatttaatgtctattaaaacagaacatcgtgagcgagctcgcgcccagggcttattcaagccaaacagctacattgacctcgcaaagacgccttgcgtggatggcaaagcaggagaatattcctgtgagaacgttgatcttcttggcttcctgagtcatcaggccatgggcagtacgacccgggaggggaatgatatctggggatggacatcagccgatggccgtgaattcggcatcgttggccaaacggacggaacggcctttgtagaagttctggacgatggcagtctgcagtatgtcggccgtctaccgacgcagacaacggcaactatttggagagatatgaaggtgattggggatcatgcctatattggatcagagtcaccgggacatggtcttcagatctttgacttgaagaagcttctcgagacggacagcaataacccgaccaatttctcgaccacggaagacctaacggcttggtacagcggttttggtagctcacacaacatcgttgcgcatgaagagactaacatgatcttcgctgtcggcacagccaggaacctatcctgcgctggcggcctgtggatgatcgatgtgtctgatcccgcgaacccgacgtcgcctggatgtgtcagtgaagacggttatgtgcacgatgcacaatgtgtgatctacaccggccccgacaaggaatacacaaaccgtgagatctgcttcaactacaacgaagacaccctcaccatcgtcgacataacagacagggcctcgccaatccagatctccaaaaccccctatgttggagcaagctacacgcaccaaggctggatagcagtctccgacatgtcctacctcctcctggacgacgaattggacgaacaagacgggacaggcgaagccgctaacggacacacaacaacgtacattttcgacattaaggacctagcgaatccgaaacatacagggacgtaccagtctcccgtgcgatcaatcgaccataaccagtatgttatcgatgggttgacataccaagctaactacgggagcggattgcgcatcgtcgatgttagctctgttaaggatgatccgacaggcaaggggttcaaacaggtgggtttctttgactgccacccagaagatgatgcccagggcggggaagttgagtttgtgggtgcttggagtgtctatccatatttccggagcgggaatattttgttgaacagtatcgagaggggtgtctattcgttgaagtacaccggaaaggcttga

SEQ ID NO: 11 - DNA, 1347 bp, synthetic construct
  source 1..1347: mol_type = other DNA
atgaaaccatcatttgtctcccttttgtccctggcttgcctcggggcagcctcccgcgagggcgctccgattatgagccatttaatgtctattaaaacagaacatcgtgagcgagctcgcgcccagggcttattcaagccaaacagctacattgacctcgcaaagacgccttgcgtggatggcaaagcaggagaatattcctgtgagaacgttgatcttcttggcttcctgagtcatcaggccatgggcagtacgacccgggaggggaatgatatctggggatggacatcagccgatggccgtgaattcggcatcgttggccaaacggacggaacggcctttgtagaagttctggacgatggcagtctgcagtatgtcggccgtctaccgacgcagacaacggcaactatttggagagatatgaaggtgattggggatcatgcctatattggatcagagtcaccgggacatggtcttcagatctttgacttgaagaagcttctcgagacggacagcaataacccgaccaatttctcgaccacggaagacctaacggcttggtacagcggttttggtagctcacacaacatcgttgcgcatgaagagactaacatgatcttcgctgtcggcacagccaggaacctatcctgcgctggcggcctgtggatgatcgatgtgtctgatcccgcgaacccgacgtcgcctggatgtgtcagtgaagacggttatgtgcacgatgcacaatgtgtgatctacaccggccccgacaaggaatacacaaaccgtgagatctgcttcaactacaacgaagacaccctcaccatcgtcgacataacagacagggcctcgccaatccagatctccaaaaccccctatgttggagcaagctacacgcaccaaggctggatagcagtctccgacatgtcctacctcctcctggacgacgaattggacgaacaagacgggacaggcgaagccgctaacggacacacaacaacgtacattttcgacattaaggacctagcgaatccgaaacatacagggacgtaccagtctcccgtgcgatcaatcgaccataaccagtatgttatcgatgggttgacataccaagctaactacgggagcggattgcgcatcgtcgatgttagctctgttaaggatgatccgacaggcaaggggttcaaacaggtgggtttctttgactgccacccagaagatgatgcccagggcggggaagttgagtttgtgggtgcttggagtgtctatccatatttccggagcgggaatattttgttgaacagtatcgagaggggtgtctattcgttgaagtacaccggaaaggcttga

SEQ ID NO: 12 - DNA, 1519 bp, Aspergillus oryzae
  source 1..1519: mol_type = genomic DNA
atgaaaccatcatttgtctcccttttgtccctggcttgcctcggggcagcctcccgcgagggcgctccgattatgagccatttaatgtctattaaaacagaacatcgtgagcgagctcgcgcccagggcttattcaagccaaacagctacattgacctcgcaaagacgccttgcgtggatggcaaagcaggagaatattcctgtgagaacgttgatcttcttggcttcctgagtcatcaggccatgggcagtacgacccgggaggggaatgatatctggggtatgttaaccatactatgcatctgttccgtggacataagatttaacatgaacaggatggacatcagccgatggccgtgaattcggcatcgttggccaaacggacggaacggcctttgtagaagttctggacgatggcagtctgcagtatgtcggccgtctaccgacgcagacaacggcaactatttggagagatatgaaggtgattggggatcatgcctatattggatcagagtcaccgggacatggtcttcagatctttgacttgaagaaggtatattatcgtaacaatattgtgctcaatacttgagtacgcccaaggctaacggagtccagcttctcgagacggacagcaataacccgaccaatttctcgaccacggaagacctaacggcttggtacagcggttttggtagctcacacaacatcgttgcgcatgaagagactaacatgatcttcgctgtcggcacagccaggaacctatcctgcgctggcggcctgtggatgatcgatgtgtctgatcccgcgaacccgacgtcgcctggatgtgtcagtgaagacggttatgtgcacgatggtaggtctctatggttcaatgggtcagctcacagtccaatactaacgcaaaccagcacaatgtgtgatctacaccggccccgacaaggaatacacaaaccgtgagatctgcttcaactacaacgaagacaccctcaccatcgtcgacataacagacagggcctcgccaatccagatctccaaaaccccctatgttggagcaagctacacgcaccaaggctggatagcagtctccgacatgtcctacctcctcctggacgacgaattggacgaacaagacgggacaggcgaagccgctaacggacacacaacaacgtacattttcgacattaaggacctagcgaatccgaaacatacagggacgtaccagtctcccgtgcgatcaatcgaccataaccagtatgttatcgatgggttgacataccaagctaactacgggagcggattgcgcatcgtcgatgttagctctgttaaggatgatccgacaggcaaggggttcaaacaggtgggtttctttgactgccacccagaagatgatgcccagggcggggaagttgagtttgtgggtgcttggagtgtctatccatatttccggagcgggaatattttgttgaacagtatcgagaggggtgtctattcgttgaagtacaccggaaaggcttga

SEQ ID NO: 13 - protein, 12 aa, synthetic construct
YGGFMRRVGRPE

SEQ ID NO: 14 - protein, 7 aa, synthetic construct
RVYIHPF